European Patent Application EP 4 431 605 A1, published September 18, 2024. Title: Genetically-modified pluripotent stem cell, immunocompetent cell derived therefrom, method of producing same and use thereof. Applicant: 株式会社ヘリオス. The sequence listing filed with the application follows.

SEQUENCE LISTING (19 sequences)

SEQ ID NO: 1 - DNA, 250 bp, Trichoplusia ni
  source 1..250: mol_type = genomic DNA
ccctagaaagataatcatattgtgacgtacgttaaagataatcatgcgtaaaattgacgcatgtgttttatcggtctgtatatcgaggtttatttattaatttgaatagatattaagttttattatatttacacttacatactaataataaattcaacaaacaatttatttatgtttatttatttattaaaaaaaaacaaaaactcaaaatttcttctataaagtaacaaaacttttaaacattctctct

SEQ ID NO: 2 - DNA, 307 bp, Trichoplusia ni
  source 1..307: mol_type = genomic DNA
tatctataacaagaaaatatatatataataagttatcacgtaagtagaacatgaaataacaatataattatcgtatgagttaaatcttaaaagtcacgtaaaagataatcatgcgtcattttgactcacgcggtcgttatagttcaaaatcagtgacacttaccgcattgacaagcacgcctcacgggagctccaagcggcgactgagatgtcctaaatgcacagcgacggattcgcgctatttagaaagagagagcaatatttcaagaatgcatgcgtcaattttacgcagactatctttctaggg

SEQ ID NO: 3 - DNA, 585 bp, synthetic construct
  misc_feature 1..585: note = IRES
  source 1..585: mol_type = other DNA
gcccctctccctcccccccccctaacgttactggccgaagccgcttggaataaggccggtgtgcgtttgtctatatgtgattttccaccatattgccgtcttttggcaatgtgagggcccggaaacctggccctgtcttcttgacgagcattcctaggggtctttcccctctcgccaaaggaatgcaaggtctgttgaatgtcgtgaaggaagcagttcctctggaagcttcttgaagacaaacaacgtctgtagcgaccctttgcaggcagcggaaccccccacctggcgacaggtgcctctgcggccaaaagccacgtgtataagatacacctgcaaaggcggcacaaccccagtgccacgttgtgagttggatagttgtggaaagagtcaaatggctctcctcaagcgtattcaacaaggggctgaaggatgcccagaaggtaccccattgtatgggatctgatctggggcctcggtgcacatgctttacatgtgtttagtcgaggttaaaaaaacgtctaggccccccgaaccacggggacgtggttttcctttgaaaaacacgatgataatatggccaca

SEQ ID NO: 4 - DNA, 479 bp, Homo sapiens
  source 1..479: mol_type = other DNA
ccgggtggcatccctgtgacccctccccagtgcctctcctggccctggaagttgccactccagtgcccaccagccttgtcctaataaaattaagttgcatcattttgtctgactaggtgtccttctataatattatggggtggaggggggtggtatggagcaaggggcaagttgggaagacaacctgtagggcctgcggggtctattgggaaccaagctggagtgcagtggcacaatcttggctcactgcaatctccgcctcctgggttcaagcgattctcctgcctcagcctcccgagttgttgggattccaggcatgcatgaccaggctcagctaatttttgtttttttggtagagacggggtttcaccatattggccaggctggtctccaactcctaatctcaggtgatctacccaccttggcctcccaaattgctgggattacaggcgtgaaccactgctcccttccctgtcctt

SEQ ID NO: 5 - DNA, 1086 bp, synthetic construct
  misc_feature 1..1086: note = Modified human CCR2B
  source 1..1086: mol_type = other DNA
atggctctgtccacatctcgttctcggtttatcagaaataccaacgagagcggtgaagaagtcaccaccttttttgattatgattacggtgctccctgtcataaatttgacgtgaagcaaattggggcccaactcctgcctccgctctactcgctggtgttcatctttggttttgtgggcaacatgctggtcgtcctcatcttaatcaactgcaaaaagctgaagtgcttgactgacatttacctgctcaacctggccatctctgatctgctttttcttattactctcccattgtgggctcactctgctgcaaatgagtgggtctttgggaatgcaatgtgcaaattattcacagggctgtatcacatcggttattttggcggaatcttcttcatcatcctcctgacaatcgatagatacctggctattgtccatgctgtgtttgctttaaaagccaggacggtcacctttggggtggtgacaagtgtgatcacctggttggtggctgtgtttgcttctgtcccaggaatcatctttactaaatgccagaaagaagattctgtttatgtctgtggcccttattttccacgaggatggaataatttccacacaataatgaggaacattttggggctggtcctgccgctgctcatcatggtcatctgctactcgggaatcctgaaaaccctgcttcggtgtcgaaacgagaagaagaggcatagggcagtgagagtcatcttcaccatcatgattgtttactttctcttctggactccctataatattgtcattctcctgaacaccttccaggaattcttcggcctgagtaactgtgaaagcaccagtcaactggaccaagccacgcaggtgacagagactcttgggatgactcactgctgcatcaatcccatcatctatgccttcgttggggagaagttcagaaggtatctctcggtgttcttccgaaagcacatcaccaagcgcttctgcaaacaatgtccagttttctacagggagacagtggatggagtgacttcaacaaacacgccttccactggggagcaggaagtctcggctggtttataa

SEQ ID NO: 6 - DNA, 297 bp, Homo sapiens
  source 1..297: mol_type = other DNA
atggccctgctactggccctcagcctgctggttctctggacttccccagccccaactctgagtggcaccaatgatgctgaagactgctgcctgtctgtgacccagaaacccatccctgggtacatcgtgaggaacttccactaccttctcatcaaggatggctgcagggtgcctgctgtagtgttcaccacactgaggggccgccagctctgtgcacccccagaccagccctgggtagaacgcatcatccagagactgcagaggacctcagccaagatgaagcgccgcagcagttaa

SEQ ID NO: 7 - DNA, 489 bp, Homo sapiens
  source 1..489: mol_type = other DNA
atgagaatttcgaaaccacatttgagaagtatttccatccagtgctacttgtgtttacttctaaacagtcattttctaactgaagctggcattcatgtcttcattttgggctgtttcagtgcagggcttcctaaaacagaagccaactgggtgaatgtaataagtgatttgaaaaaaattgaagatcttattcaatctatgcatattgatgctactttatatacggaaagtgatgttcaccccagttgcaaagtaacagcaatgaagtgctttctcttggagttacaagttatttcacttgagtccggagatgcaagtattcatgatacagtagaaaatctgatcatcctagcaaacaacagtttgtcttctaatgggaatgtaacagaatctggatgcaaagaatgtgaggaactggaggaaaaaaatattaaagaatttttgcagagttttgtacatattgtccaaatgttcatcaacacttcttaa

SEQ ID NO: 8 - DNA, 804 bp, Homo sapiens
  source 1..804: mol_type = other DNA
atggccccgcggcgggcgcgcggctgccggaccctcggtctcccggcgctgctactgctgctgctgctccggccgccggcgacgcggggcatcacgtgccctccccccatgtccgtggaacacgcagacatctgggtcaagagctacagcttgtactccagggagcggtacatttgtaactctggtttcaagcgtaaagccggcacgtccagcctgacggagtgcgtgttgaacaaggccacgaatgtcgcccactggacaacccccagtctcaaatgcattagagaccctgccctggttcaccaaaggccagcgccaccctccacagtaacgacggcaggggtgaccccacagccagagagcctctccccttctggaaaagagcccgcagcttcatctcccagctcaaacaacacagcggccacaacagcagctattgtcccgggctcccagctgatgccttcaaaatcaccttccacaggaaccacagagataagcagtcatgagtcctcccacggcaccccctctcagacaacagccaagaactgggaactcacagcatccgcctcccaccagccgccaggtgtgtatccacagggccacagcgacaccactgtggctatctccacgtccactgtcctgctgtgtgggctgagcgctgtgtctctcctggcatgctacctcaagtcaaggcaaactcccccgctggccagcgttgaaatggaagccatggaggctctgccggtgacttgggggaccagcagcagagatgaagacttggaaaactgctctcaccacctataa

SEQ ID NO: 9 - DNA, 618 bp, Homo sapiens
  source 1..618: mol_type = other DNA
atggccccgcggcgggcgcgcggctgccggaccctcggtctcccggcgctgctactgctgctgctgctccggccgccggcgacgcggggcatcacgtgccctccccccatgtccgtggaacacgcagacatctgggtcaagagctacagcttgtactccagggagcggtacatttgtaactctggtttcaagcgtaaagccggcacgtccagcctgacggagtgcgtgttgaacaaggccacgaatgtcgcccactggacaacccccagtctcaaatgcattagagaccctgccctggttcaccaaaggccagcgccaccctccacagtaacgacggcaggggtgaccccacagccagagagcctctccccttctggaaaagagcccgcagcttcatctcccagctcaaacaacacagcggccacaacagcagctattgtcccgggctcccagctgatgccttcaaaatcaccttccacaggaaccacagagataagcagtcatgagtcctcccacggcaccccctctcagacaacagccaagaactgggaactcacagcatccgcctcccaccagccgccaggtgtgtatccacagggccacagcgacaccacttaa

SEQ ID NO: 10 - DNA, 405 bp, synthetic construct
  misc_feature 1..405: note = IL-2 signal peptide-fused IL-15
  source 1..405: mol_type = other DNA
atgtacaggatgcaactcctgtcttgcattgcactaagtcttgcacttgtcacaaacagtaactgggtgaatgtaataagtgatttgaaaaaaattgaagatcttattcaatctatgcatattgatgctactttatatacggaaagtgatgttcaccccagttgcaaagtaacagcaatgaagtgctttctcttggagttacaagttatttcacttgagtccggagatgcaagtattcatgatacagtagaaaatctgatcatcctagcaaacaacagtttgtcttctaatgggaatgtaacagaatctggatgcaaagaatgtgaggaactggaggaaaaaaatattaaagaatttttgcagagttttgtacatattgtccaaatgttcatcaacacttcttaa

SEQ ID NO: 11 - DNA, 772 bp, synthetic construct
  misc_feature 1..772: note = human CD16a F176V natural variant
  source 1..772: mol_type = other DNA
atgtggcagctgctcctcccaactgctctgctacttctagtttcagctggcatgcggactgaagatctcccaaaggctgtggtgttcctggagcctcaatggtacagggtgctcgagaaggacagtgtgactctgaagtgccagggagcctactcccctgaggacaattccacacagtggtttcacaatgagagcctcatctcaagccaggcctcgagctacttcattgacgctgccacagtcgacgacagtggagagtacaggtgccagacaaacctctccaccctcagtgacccggtgcagctagaagtccatatcggctggctgttgctccaggcccctcggtgggtgttcaaggaggaagaccctattcacctgaggtgtcacagctggaagaacactgctctgcataaggtcacatatttacagaatggcaaaggcaggaagtattttcatcataattctgacttctacattccaaaagccacactcaaagacagcggctcctacttctgcagggggcttgtcgggagtaaaaatgtgtcttcagagactgtgaacatcaccatcactcaaggtttggcagtgtcaaccatctcatcattctttccacctgggtaccaagtctctttctgcttggtgatggtactcctttttgcagtggacacaggactatatttctctgtgaagacaaacattcgaagctcaacaagagactggaaggaccataaatttaaatggagaaaggaccctcaagacaaatgagggctaa

SEQ ID NO: 12 - DNA, 651 bp, synthetic construct
  misc_feature 1..651: note = modified human NKG2D
  source 1..651: mol_type = other DNA
atggggtggattcgtggtcggaggtctcgacacagctgggagatgagtgaatttcataattataacttggatctgaagaagagtgatttttcaacacgatggcaaaagcaaagatgtccagtagtcaaaagcaaatgtagagaaaatgcatctccattttttttctgctgcttcatcgctgtagccatgggaatccgtttcattattatggtaacaatatggagtgctgtattcctaaactcattattcaaccaagaagttcaaattcccttgaccgaaagttactgtggcccatgtcctaaaaactggatatgttacaaaaataactgctaccaattttttgatgagagtaaaaactggtatgagagccaggcttcttgtatgtctcaaaatgccagccttctgaaagtatacagcaaagaggaccaggatttacttaaactggtgaagtcatatcattggatgggactggtacacattccaacaaatggatcttggcagtgggaagatggctccattctctcacccaacctactaacaataattgaaatgcagaagggagactgtgcactctatgcctcgagctttaaaggctatatagaaaactgttcaactccaaatacgtacatctgcatgcaaaggactgtgtaa

SEQ ID NO: 13 - DNA, 1416 bp, synthetic construct
  misc_feature 1..1416: note = NKG2D-CAR
  source 1..1416: mol_type = other DNA
atggccttaccagtgaccgccttgctcctgccgctggccttgctgctccacgccgccaggccgttattcaaccaagaagttcaaattcccttgaccgaaagttactgtggcccatgtcctaaaaactggatatgttacaaaaataactgctaccaattttttgatgagagtaaaaactggtatgagagccaggcttcttgtatgtctcaaaatgccagccttctgaaagtatacagcaaagaggaccaggatttacttaaactggtgaagtcatatcattggatgggactagtacacattccaacaaatggatcttggcagtgggaagatggctccattctctcacccaacctactaacaataattgaaatgcagaagggagactgtgcactctatgcctcgagctttaaaggctatatagaaaactgttcaactccaaatacgtacatctgcatgcaaaggactgtgttcgtgccggtcttcctgccagcgaagcccaccacgacgccagcgccgcgaccaccaacaccggcgcccaccatcgcgtcgcagcccctgtccctgcgcccagaggcgtgccggccagcggcggggggcgcagtgcacacgagggggctggacttcgcctgtgatatctacatctgggcgcccttggccgggacttgtggggtccttctcctgtcactggttatcaccctttactgcaaccacaggaactggaggagaaagaggaaggagaagcagtcagagaccagtcccaaggaatttttgacaatttacgaagatgtcaaggatctgaaaaccaggagaaatcacgagcaggagcagacttttcctggaggggggagcaccatctactctatgatccagtcccagtcttctgctcccacgtcacaagaacctgcatatacattatattcattaattcagccttccaggaagtctggatccaggaagaggaaccacagcccttccttcaatagcactatctatgaagtgattggaaagagtcaacctaaagcccagaaccctgctcgattgagccgcaaagagctggagaactttgatgtttattccagagtgaagttcagcaggagcgcagacgcccccgcgtaccagcagggccagaaccagctctataacgagctcaatctaggacgaagagaggagtacgatgttttggacaagagacgtggccgggaccctgagatggggggaaagccgagaaggaagaaccctcaggaaggcctgtacaatgaactgcagaaagataagatggcggaggcctacagtgagattgggatgaaaggcgagcgccggaggggcaaggggcacgatggcctttaccagggtctcagtacagccaccaaggacacctacgacgcccttcacatgcaggccctgccccctcgctaa

SEQ ID NO: 14 - DNA, 282 bp, synthetic construct
  misc_feature 1..282: note = Modified human DAP10
  source 1..282: mol_type = other DNA
atgatccatctgggtcacatcctcttcctgcttttgctcccagtggctgcagctcagacgactccaggagagagatcatcactccctgccttttaccctggcacttcaggctcttgttccggatgtgggtccctctctctgccgctcctggcaggcctcgtggctgctgatgcggtggcatcgctgctcatcgtgggagcagtgtttctttgtgcaagacctaggagatctccagctcaagaagatggcaaagtctacatcaacatgccaggcaggggctga

SEQ ID NO: 15 - DNA, 600 bp, synthetic construct
  misc_feature 1..600: note = Puromycin-resistant gene
  source 1..600: mol_type = other DNA
atgaccgaatataaacctacggttagattggcgacaagggacgacgtgcctagagctgtacgcacactggcagccgcatttgcggactacccggcaacacgacacaccgtggaccctgatcgccacatagagcgggtcactgaactccaggaattgtttctcacccgagtaggccttgacattggcaaggtatgggtcgcggacgacggtgccgccgttgctgtctggactaccccggaaagcgtagaagctggagctgtattcgcagagatcggtccaaggatggcagagctttctggctccagacttgccgcccaacaacagatggaaggacttctggcgccccataggccgaaagagcctgcgtggtttttggctacagttggcgtttccccagatcatcaaggtaaagggctcggatctgccgtggtgcttcctggggttgaggcagctgagagggccggtgttcctgcgttccttgagacatccgctcctcgcaacttgcctttctatgaaaggctgggttttactgttacggccgatgtagaagtgccagaaggaccacgcacctggtgcatgactagaaagcctggggcatga

SEQ ID NO: 16 - DNA, 1038 bp, synthetic construct
  misc_feature 1..1038: note = Hygromycin resistant gene
  source 1..1038: mol_type = other DNA
atgaaaaagcctgaactcaccgcgacgtctgtcgagaagtttctgatcgaaaagttcgacagcgtctccgacctgatgcagctctcggagggcgaagaatctcgtgctttcagcttcgatgtaggagggcgtggatatgtcctgcgggtaaatagctgcgccgatggtttctacaaagatcgttatgtttatcggcactttgcatcggccgcgctcccgattccggaagtgcttgacattggggaattcagcgagagcctgacctattgcatctcccgccgtgcacagggtgtcacgttgcaagacctgcctgaaaccgaactgcccgctgttctgcagccggtcgcggaggccatggatgcgatcgctgcggccgatcttagccagacgagcgggttcggcccattcggaccgcaaggaatcggtcaatacactacatggcgtgatttcatatgcgcgattgctgatccccatgtgtatcactggcaaactgtgatggacgacaccgtcagtgcgtccgtcgcgcaggctctcgatgagctgatgctttgggccgaggactgccccgaagtccggcacctcgtgcacgcggatttcggctccaacaatgtcctgacggacaatggccgcataacagcggtcattgactggagcgaggcgatgttcggggattcccaatacgaggtcgccaacatcttcttctggaggccgtggttggcttgtatggagcagcagacgcgctacttcgagcggaggcatccggagcttgcaggatcgccgcggctccgggcgtatatgctccgcattggtcttgaccaactctatcagagcttggttgacggcaatttcgatgatgcagcttgggcgcagggtcgatgcgacgcaatcgtccgatccggagccgggactgtcgggcgtacacaaatcgcccgcagaagcgcggccgtctggaccgatggctgtgtagaagtactcgccgatagtggaaaccgacgccccagcactcgtggggatcgggagatgggggaggctaactga

SEQ ID NO: 17 - DNA, 375 bp, synthetic construct
  misc_feature 1..375: note = Zeocin-resistant gene
  source 1..375: mol_type = other DNA
atggcaaagctcacaagcgcagtccctgtgttgacagcaagagatgtcgccggagcagtcgagttttggactgataggttgggattcagcagggacttcgtcgaagatgactttgctggcgtcgtgagagacgatgtgactctgttcatcagcgcagtccaggatcaggttgtccctgacaacaccctcgcttgggtctgggttaggggactcgacgaactctacgcagaatggagcgaagtcgtgtccaccaactttcgggatgcctccggccctgctatgactgagatcggagaacagccttggggaagggaatttgcactgagagatcctgccggaaactgcgtccacttcgtcgctgaagagcaagattga

SEQ ID NO: 18 - DNA, 804 bp, synthetic construct
  misc_feature 1..804: note = Neomycin-resistant gene
  source 1..804: mol_type = other DNA
atgggatctgccatcgaacaggatgggctccatgcaggatctccagccgcatgggtggaaaggttgttcggatacgactgggctcagcaaactatcggatgctctgatgcagcggtttttcgcctctccgctcagggacgccctgtacttttcgtcaagacagatttgagcggcgcactcaatgaactccaggacgaagctgctagactgtcctggttggctaccactggggttccctgtgctgctgtcttggacgttgttacagaagctggaagagattggctcctgctcggagaagtgcctggacaggacctcctctccagccacctcgcacctgccgagaaagtcagcatcatggcagatgctatgcgccgccttcataccctcgatcccgcaacatgcccattcgatcaccaggccaagcacaggatagagagagcacgcactagaatggaagctggattggtcgatcaagatgatctcgacgaagaacatcagggccttgctcctgccgaattgttcgctcggctcaaagccagaatgcccgatggcgaggatctggtcgttacacatggcgacgcatgtctcccaaacatcatggttgagaacggacggttctctggctttatcgactgcggacggctgggagtcgcagatagataccaagacattgcactggctaccagagatatagcagaggaactcggcggagagtgggcagatagatttctcgttctgtatggtattgctgcacccgatagccaaagaatcgccttttatagactcctggatgagtttttctga

SEQ ID NO: 19 - DNA, 1785 bp, synthetic construct
  misc_feature 1..1785: note = PBase
  source 1..1785: mol_type = other DNA
atgggaagctccctggacgatgaacatatcctctccgctctgctccaaagcgatgacgaactggtgggcgaggattccgactctgagatttctgaccatgtcagcgaggacgatgtgcagtccgatactgaagaggcatttatcgacgaggtgcatgaagtccagcccacttcctctggaagcgaaatcctggacgagcagaatgtcatcgaacagcctggctcctctctcgcttccaacagaatcctgaccctccctcagaggacaatcagaggcaagaacaagcattgctggtctacaagcaaatccaccaggagaagccgggtgtctgccctcaatatcgtcagaagccaaaggggacccacccggatgtgtaggaacatttacgatcctctgctctgcttcaagctgtttttcactgacgagatcatttctgaaattgtgaagtggacaaacgccgaaatctctctcaagagaagggaaagcatgacaggggctacattcagggacacaaatgaggatgaaatttacgccttctttggcattctggtgatgacagcagtcagaaaagataatcacatgagcacagatgatctcttcgacagatccctgagcatggtgtatgtctctgtgatgtccagagatcggttcgattttctcattagatgcctgcggatggacgataaatccatcaggcccactctcagagagaatgatgtgttcacccctgtgcggaagatttgggatctgttcatccaccagtgcattcaaaattacacccccggcgctcatctcacaatcgacgaacaactcctgggatttcggggcagatgtcccttcagaatgtatattcctaataagccaagcaagtacgggatcaaaattctgatgatgtgtgactctggaaccaagtatatgattaacggaatgccttatctcggcagagggacccaaactaacggcgtgccactcggcgaatactatgtcaaagagctgtccaaacctgtccacggaagctgtagaaatatcacctgcgataactggtttacatccattcccctcgccaagaacctgctccaagaaccttacaagctgaccattgtcggcactgtcaggtccaacaagagggagattccagaagtgctcaagaactccagaagcaggccagtcggcacatccatgttctgtttcgacggaccactgactctcgtgtcttacaagcccaaacctgctaagatggtctatctgctcagctcctgtgatgaggacgcctctattaacgagagcaccggcaagccacaaatggtgatgtactataaccagaccaaggggggagtcgatactctcgaccagatgtgttccgtgatgacatgctccagaaagactaatcggtggcctatggctctcctgtatggcatgattaacattgcctgtatcaacagcttcatcatttatagccacaacgtgtcctctaagggagaaaaggtccaaagcagaaagaaattcatgcggaacctgtatatgagcctcacctcctcttttatgcggaagaggctggaggcacctactctcaaaagatacctgagggataacatcagcaacattctccctaatgaggtccccggaacatccgacgattctactgaggaacctgtgatgaagaaacggacctattgcacatactgtcctagcaagatcagaaggaaggcaaatgcttcctgcaagaaatgtaagaaggtcatttgtagagaacataacattgatatgtgtcagagctgcttctaa